European Patent Application EP 4 796 128 A1, published August 26, 2026. Title: Anti-c-MET Antibody-Drug Conjugates Containing Camptothecin Derivatives. Applicant: Celltrion, Inc. The sequence listing filed with the application follows.

SEQUENCE LISTING (14 sequences)

SEQ ID NO: 1 - protein, 8 aa, synthetic construct
GYIFTAYT

SEQ ID NO: 2 - protein, 8 aa, synthetic construct
IKPNNGLA

SEQ ID NO: 3 - protein, 11 aa, synthetic construct
ARSEITTEFDY

SEQ ID NO: 4 - protein, 10 aa, synthetic construct
ESVDSYANSF

SEQ ID NO: 5 - skipped

SEQ ID NO: 6 - protein, 9 aa, synthetic construct
QQSKEDPLT

SEQ ID NO: 7 - protein, 118 aa, synthetic construct
QVQLVQSGAEVKKPGASVKVSCKASGYIFTAYTMHWVRQAPGQGLEWMGWIKPNNGLANYAQKFQGRVTMTRDTSISTAYMELSRLRSDDTAVYYCARSEITTEFDYWGQGTLVTVSS

SEQ ID NO: 8 - protein, 111 aa, synthetic construct
DIVMTQSPDSLAVSLGERATINCKSSESVDSYANSFLHWYQQKPGQPPKLLIYRASTRESGVPDRFSGSGSGTDFTLTISSLQAEDVAVYYCQQSKEDPLTFGGGTKVEIK

SEQ ID NO: 9 - protein, 448 aa, synthetic construct
QVQLVQSGAEVKKPGASVKVSCKASGYIFTAYTMHWVRQAPGQGLEWMGWIKPNNGLANYAQKFQGRVTMTRDTSISTAYMELSRLRSDDTAVYYCARSEITTEFDYWGQGTLVTVSSASTKGPSVFPLAPSSKSTSGGTAALGCLVKDYFPEPVTVSWNSGALTSGVHTFPAVLQSSGLYSLSSVVTVPSSSLGTQTYICNVNHKPSNTKVDKKVEPKSCDKTHTCPPCPAPELLGGPSVFLFPPKPKDTLMISRTPEVTCVVVDVSHEDPEVKFNWYVDGVEVHNAKTKPREEQYNSTYRVVSVLTVLHQDWLNGKEYKCKVSNKALPAPIEKTISKAKGQPREPQVYTLPPSRDELTKNQVSLTCLVKGFYPSDIAVEWESNGQPENNYKTTPPVLDSDGSFFLYSKLTVDKSRWQQGNVFSCSVMHEALHNHYTQKSLSLSPGK

SEQ ID NO: 10 - protein, 218 aa, synthetic construct
DIVMTQSPDSLAVSLGERATINCKSSESVDSYANSFLHWYQQKPGQPPKLLIYRASTRESGVPDRFSGSGSGTDFTLTISSLQAEDVAVYYCQQSKEDPLTFGGGTKVEIKRTVAAPSVFIFPPSDEQLKSGTASVVCLLNNFYPREAKVQWKVDNALQSGNSQESVTEQDSKDSTYSLSSTLTLSKADYEKHKVYACEVTHQGLSSPVTKSFNRGEC

SEQ ID NO: 11 - protein, 449 aa, synthetic construct
EVQLVQSGGGLIQPGGSLRLSCAASEFIVSSNYMTWVRQAPGKGLEWVSIIYPGGSTYYADSVKGRFTISRDNSKNTLYLRMNSLRAEDTAVYYCARDLPLTGTTLDYWGQGTLVTVSSASTKGPSVFPLAPSSKSTSGGTAALGCLVKDYFPEPVTVSWNSGALTSGVHTFPAVLQSSGLYSLSSVVTVPSSSLGTQTYICNVNHKPSNTKVDKRVEPKSCDKTHTCPPCPAPELLGGPSVFLFPPKPKDTLMISRTPEVTCVVVDVSHEDPEVKFNWYVDGVEVHNAKTKPREEQYNSTYRVVSVLTVLHQDWLNGKEYKCKVSNKALPAPIEKTISKAKGQPREPQVYTLPPSRDELTKNQVSLTCLVKGFYPSDIAVEWESNGQPENNYKTTPPVLDSDGSFFLYSKLTVDKSRWQQGNVFSCSVMHEALHNHYTQKSLSLSPGK

SEQ ID NO: 12 - protein, 214 aa, synthetic construct
ELVLTQSPSSLSASVGDRVTITCRASQSISSYLNWYQQKPGKAPKLLIYAASSLQSGVPSRFSGSGSGTDFTLTISSLQPEDFATYYCQQSYSTPLTFGGGTKLEIKRTVAAPSVFIFPPSDEQLKSGTASVVCLLNNFYPREAKVQWKVDNALQSGNSQESVTEQDSKDSTYSLSSTLTLSKADYEKHKVYACEVTHQGLSSPVTKSFNRGEC

SEQ ID NO: 13 - protein, 475 aa, synthetic construct
MDWTWSILFLVAAATGAHSQVQLVQSGAEVKKPGASVKVSCKTSGYSFSTYGVSWVRQAPGQGPEWVGWISAYTGITDYAQKFQGRVTLTTDATTATAFLDLRSLRPDDTATYFCARDKVQGRVEVGSGGRHDYWGQGTLVIVSSASTKGPSVFPLAPSSKSTSGGTAALGCLVKDYFPEPVTVSWNSGALTSGVHTFPAVLQSSGLYSLSSVVTVPSSSLGTQTYICNVNHKPSNTKVDKKVEPKSCDKTHTCPPCPAPELLGGPSVFLFPPKPKDTLMISRTPEVTCVVVDVSHEDPEVKFNWYVDGVEVHNAKTKPREEQYNSTYRVVSVLTVLHQDWLNGKEYKCKVSNKALPAPIEKTISKAKGQPREPQVYTLPPSRDELTKNQVSLTCLVKGFYPSDIAVEWESNGQPENNYKTTPPVLDSDGSFFLYSKLTVDKSRWQQGNVFSCSVMHEGLHNHYTQKSLSLSPGK

SEQ ID NO: 14 - protein, 235 aa, synthetic construct
METPAQLLFLLLLWLPDTTGEVVLTQSPGTLALPPGERATLSCRASHRVGSTYIAWYQQKSGQAPRRLIYGASNRATDIPDRFSGSGSGTDFTLTIRRLEPEDSAVYYCQQFSVSPWTFGQGTRVEIKRTVAAPSVFIFPPSDEQLKSGTASVVCLLNNFYPREAKVQWKVDNALQSGNSQESVTEQDSKDSTYSLSSTLTLSKADYEKHKVYACEVTHQGLSSPVTKSFNRGEC